European Patent Specification EP 3 505 536 B1, published August 7, 2024. Title: Antikörper gegen das Prostata-spezifische Stammzellantigen und dessen Verwendung. Applicant: AvenCell Europe GmbH. Application EP 18 207 370.0. The sequence listing filed with the application follows.

SEQUENCE LISTING (172 sequences)

SEQ ID NO: 1 - protein, 11 aa, Mus musculus
GTSQDINNYLN

SEQ ID NO: 2 - protein, 7 aa, Mus musculus
YTSRLHS

SEQ ID NO: 3 - protein, 9 aa, Mus musculus
QQSKTLPWT

SEQ ID NO: 4 - protein, 5 aa, Mus musculus
SYSMS

SEQ ID NO: 5 - protein, 17 aa, Mus musculus
YINDSGGSTFYPDTVKG

SEQ ID NO: 6 - protein, 13 aa, Mus musculus
RMYYGNSHWHFDV

SEQ ID NO: 7 - DNA, 33 bp, Mus musculus
gggacaagtcaggacattaacaattatttaaac

SEQ ID NO: 8 - DNA, 33 bp, Homo sapiens
ggtacatcccaagacatcaataattatctcaac

SEQ ID NO: 9 - DNA, 21 bp, Mus musculus
tacacatcaagattacactcg

SEQ ID NO: 10 - DNA, 21 bp, Homo sapiens
tacacatccaggctgcattcc

SEQ ID NO: 11 - DNA, 27 bp, Mus musculus
caacagtctaagacgcttccgtggacg

SEQ ID NO: 12 - DNA, 27 bp, Homo sapiens
cagcagtcaaagacattaccatggaca

SEQ ID NO: 13 - DNA, 15 bp, Mus musculus
tcctattccatgtct

SEQ ID NO: 14 - DNA, 15 bp, Homo sapiens
agttactctatgtca

SEQ ID NO: 15 - DNA, 51 bp, Mus musculus
tacattaatgatagtggtggtagcaccttttatccagacactgtgaagggc

SEQ ID NO: 16 - DNA, 51 bp, Homo sapiens
tacattaatgattcaggtggaagtacattctatccggacacggttaaaggt

SEQ ID NO: 17 - DNA, 39 bp, Mus musculus
cggatgtactacggtaatagccactggcacttcgatgtc

SEQ ID NO: 18 - DNA, 39 bp, Homo sapiens
cgtatgtattatggcaatagtcactggcactttgacgtc

SEQ ID NO: 19 - DNA, 348 bp, Mus musculus
gatattgtgatgacacagtctacatcctccctgtctgcctctctgggagacagagtcaccatcaattgcgggacaagtcaggacattaacaattatttaaactggtatcagcagaaaccagatggaagtgttaaactcctgatctactacacatcaagattacactcgggagtcccatccaggttcagtggcagtgggtctggaacagattattctctcaccattagcaacctggagcaaggggatattgccacttacttctgccaacagtctaagacgcttccgtggacgttcggtggaggcaccaagctggaactcaaacgggctgatgctgcaccaactgtatcc

SEQ ID NO: 20 - protein, 116 aa, Mus musculus
DIVMTQSTSSLSASLGDRVTINCGTSQDINNYLNWYQQKPDGSVKLLIYYTSRLHSGVPSRFSGSGSGTDYSLTISNLEQGDIATYFCQQSKTLPWTFGGGTKLELKRADAAPTVS

SEQ ID NO: 21 - DNA, 363 bp, Mus musculus
gtacagctgcaggagtcagggggagttttagtgcagcctggagggtccctgaaactctcctgtgcagcctctggattcactttcagttcctattccatgtcttggattcgccagactccagacaggaggctggagtgggtcgcatacattaatgatagtggtggtagcaccttttatccagacactgtgaagggccgattctccatctccagagacaatgccaagaacaccctgtacctccaaataagcagactgaggtctggggacacggccatttattactgttcaagacggatgtactacggtaatagccactggcacttcgatgtctggggcgcagggaccacggtcaccgtctcctca

SEQ ID NO: 22 - protein, 121 aa, Mus musculus
VQLQESGGVLVQPGGSLKLSCAASGFTFSSYSMSWIRQTPDRRLEWVAYINDSGGSTFYPDTVKGRFSISRDNAKNTLYLQISRLRSGDTAIYYCSRRMYYGNSHWHFDVWGAGTTVTVSS

SEQ ID NO: 23 - DNA, 321 bp, Homo sapiens
gatatccagatgactcaaagtcctagttccctgtctgcatcagtgggagaccgggtgaccattacatgcggtacatcccaagacatcaataattatctcaactggtatcagcagaagccaggcaaagttcctaagttattaatctactacacatccaggctgcattccggggtgccctcccgcttttcgggctccgggtcgggaaccgactttaccctaaccatatcttccctgcagcctgaagacgttgcaacgtactattgtcagcagtcaaagacattaccatggacatttggtggtgggacgcaactcactgtactt

SEQ ID NO: 24 - protein, 107 aa, Homo sapiens
DIQMTQSPSSLSASVGDRVTITCGTSQDINNYLNWYQQKPGKVPKLLIYYTSRLHSGVPSRFSGSGSGTDFTLTISSLQPEDVATYYCQQSKTLPWTFGGGTQLTVL

SEQ ID NO: 25 - DNA, 366 bp, Homo sapiens
caggtgcagctagtggagtccggtggcggcctcgttaagccgggcggatcgctgcgcctttcatgtgccgcatcaggattcacattctccagttactctatgtcatggattcggcaggcacctggcaagggattggaatgggtctcgtacattaatgattcaggtggaagtacattctatccggacacggttaaaggtagatttaccatcagccgtgataacgcgaagaatagcttgtacttacagatgaatagcctgcgtgcagaggatactgctgtatattattgcgctcgacgtatgtattatggcaatagtcactggcactttgacgtctggggccagggcacgacagttactgtctcttcg

SEQ ID NO: 26 - protein, 122 aa, Homo sapiens
QVQLVESGGGLVKPGGSLRLSCAASGFTFSSYSMSWIRQAPGKGLEWVSYINDSGGSTFYPDTVKGRFTISRDNAKNSLYLQMNSLRAEDTAVYYCARRMYYGNSHWHFDVWGQGTTVTVSS

SEQ ID NO: 27 - protein, 11 aa, Mus musculus
RTSQDISNYLN

SEQ ID NO: 28 - protein, 7 aa, Mus musculus
YTLKLNS

SEQ ID NO: 29 - protein, 9 aa, Mus musculus
QQSKTLPWT

SEQ ID NO: 30 - protein, 5 aa, Mus musculus
SYTMS

SEQ ID NO: 31 - protein, 17 aa, Mus musculus
YIHNGGGHTYYPDTIKG

SEQ ID NO: 32 - protein, 13 aa, Mus musculus
RMYYGNSHWYFDV

SEQ ID NO: 33 - DNA, 33 bp, Mus musculus
aggacaagccaggacattagcaactatttaaac

SEQ ID NO: 34 - DNA, 33 bp, Homo sapiens
cggacctcacaagacatcagcaactatctgaat

SEQ ID NO: 35 - DNA, 21 bp, Mus musculus
tacacattaaaattaaattca

SEQ ID NO: 36 - DNA, 21 bp, Homo sapiens
tacacattaaaactaaattcc

SEQ ID NO: 37 - DNA, 27 bp, Mus musculus
caacagagtaaaacacttccgtggacg

SEQ ID NO: 38 - DNA, 27 bp, Homo sapiens
cagcagtccaaaaccctgccttggacc

SEQ ID NO: 39 - DNA, 15 bp, Mus musculus
tcctataccatgtct

SEQ ID NO: 40 - DNA, 15 bp, Homo sapiens
agctatacaatgtct

SEQ ID NO: 41 - DNA, 51 bp, Mus musculus
tacattcataatggtggtggtcacacctactatccagacaccataaagggc

SEQ ID NO: 42 - DNA, 51 bp, Homo sapiens
tacatccataatggaggcggtcacacctactatcctgacactatcaaagga

SEQ ID NO: 43 - DNA, 39 bp, Mus musculus
cgaatgtactacggtaatagccactggtacttcgatgtc

SEQ ID NO: 44 - DNA, 39 bp, Homo sapiens
cgtatgtactacgggaacagccactggtacttcgacgtg

SEQ ID NO: 45 - DNA, 348 bp, Mus musculus
gatattgtgatgacacagtctccatcctccctgtctgcctctctgggcgacagagtcaccatcaattgcaggacaagccaggacattagcaactatttaaactggtatcagctgacaccagatggaactgttaaactcctgatctactacacattaaaattaaattcaggagtcccatcaaggttcagtggcagtgggtctgggacagattattctctcaccattaacaacctggagaaagaggattttgccacttatttttgccaacagagtaaaacacttccgtggacgttcggtggaggcaccaagctggaaatcaagcgggctgatgctgcaccaactgtatcc

SEQ ID NO: 46 - protein, 116 aa, Mus musculus
DIVMTQSPSSLSASLGDRVTINCRTSQDISNYLNWYQLTPDGTVKLLIYYTLKLNSGVPSRFSGSGSGTDYSLTINNLEKEDFATYFCQQSKTLPWTFGGGTKLEIKRADAAPTVS

SEQ ID NO: 47 - DNA, 363 bp, Mus musculus
caggtgaagctgcaggagtctgggggaggtttagtgcagcctggagggtccctgaaactctcctgtgtagcctctggattcactttcagttcctataccatgtcttgggttcgccggactccagagaagaggctggaatgggtcgcatacattcataatggtggtggtcacacctactatccagacaccataaagggccgattcaccatctccagagacaatgccaagaacaccctgttcctggaaatgagcagtctgaagtctgaagacacggccatgtattactgtacaagacgaatgtactacggtaatagccactggtacttcgatgtctggggcgcagggacctcggtcaccgtctcc

SEQ ID NO: 48 - protein, 121 aa, Mus musculus
QVKLQESGGGLVQPGGSLKLSCVASGFTFSSYTMSWVRRTPEKRLEWVAYIHNGGGHTYYPDTIKGRFTISRDNAKNTLFLEMSSLKSEDTAMYYCTRRMYYGNSHWYFDVWGAGTSVTVS

SEQ ID NO: 49 - DNA, 321 bp, Homo sapiens
gatatccagatgacgcaatcaccgagttctctatccgcgtcggttggcgacagagtgactatcacatgtcggacctcacaagacatcagcaactatctgaattggtatcaacaaaagccaggcaaggctcccaagctattaatttattacacattaaaactaaattccggtgtcccatccagattctcgggtagcgggtcggggacggattttaccttcacgatatcctccctccagcctgaggacatcgccacgtactactgccagcagtccaaaaccctgccttggaccttcggtggagggaccaaagtcgaaattaag

SEQ ID NO: 50 - protein, 107 aa, Homo sapiens
DIQMTQSPSSLSASVGDRVTITCRTSQDISNYLNWYQQKPGKAPKLLIYYTLKLNSGVPSRFSGSGSGTDFTFTISSLQPEDIATYYCQQSKTLPWTFGGGTKVEIK

SEQ ID NO: 51 - DNA, 366 bp, Homo sapiens
gaggtacagcttgttgaatctggaggtggcctggttcagcccggcggctcactaaggcttagttgtgccgcttcagggttcacattttccagctatacaatgtcttgggtccgacaggcaccgggaaaaggactggagtgggtgagctacatccataatggaggcggtcacacctactatcctgacactatcaaaggaaggttcactatcagtcgagataatgcgaagaactcactctacctacagatgaacagcctgcgcgccgaagacaccgctgtatactattgcgcacgccgtatgtactacgggaacagccactggtacttcgacgtgtggggtcaaggtacgaccgttaccgtgtcttcc

SEQ ID NO: 52 - protein, 122 aa, Homo sapiens
EVQLVESGGGLVQPGGSLRLSCAASGFTFSSYTMSWVRQAPGKGLEWVSYIHNGGGHTYYPDTIKGRFTISRDNAKNSLYLQMNSLRAEDTAVYYCARRMYYGNSHWYFDVWGQGTTVTVSS

SEQ ID NO: 53 - DNA, 318 bp, Homo sapiens
gaaattgtgttgacacagtctccagccaccctgtctttgtctccaggggaaagagccaccctctcctgcagtgccagttcaagtgtaagttacatgcactggtaccaacagaaacctggccaggctcccaggctcctcatctatgacacatccaaactggcttctggcatcccagccaggttcagtggcagtgggtctgggacagacttcactctcaccatcagcagcctagagcctgaagattttgcagtttattactgtcagcagtggagtagtaacccgctcacgttcggcggagggaccaaggtggagatcaaa

SEQ ID NO: 54 - DNA, 30 bp, Homo sapiens
agtgccagttcaagtgtaagttacatgcac

SEQ ID NO: 55 - DNA, 21 bp, Homo sapiens
gacacatccaaactggcttct

SEQ ID NO: 56 - DNA, 27 bp, Homo sapiens
cagcagtggagtagtaacccgctcacg

SEQ ID NO: 57 - protein, 106 aa, Homo sapiens
EIVLTQSPATLSLSPGERATLSCSASSSVSYMHWYQQKPGQAPRLLIYDTSKLASGIPARFSGSGSGTDFTLTISSLEPEDFAVYYCQQWSSNPLTFGGGTKVEIK

SEQ ID NO: 58 - protein, 10 aa, Homo sapiens
SASSSVSYMH

SEQ ID NO: 59 - protein, 7 aa, Homo sapiens
DTSKLAS

SEQ ID NO: 60 - protein, 9 aa, Homo sapiens
QQWSSNPLT

SEQ ID NO: 61 - DNA, 351 bp, Homo sapiens
caggttcagctggtgcagtctggagctgaggtgaagaagcctggggcctcagtgaaggtctcctgtaaggcttctggttacacctttaccaaatatgttatacattgggtgcgacaggcccctggacaagggcttgagtggatgggatatattaatccttacaatgatgttagtaagtacaatgagaagttcagaggcagagtcaccatgaccacagacacatccacgagcacagcctacatggagctgaggagcctgagatctgacgacacggccgtgtattactgtgcgagaaataaggattactatcctatggactactggggccaagggaccacggtcaccgtctcg

SEQ ID NO: 62 - DNA, 15 bp, Mus musculus
aaatatgttatacat

SEQ ID NO: 63 - DNA, 51 bp, Mus musculus
tatattaatccttacaatgatgttagtaagtacaatgagaagttcagaggc

SEQ ID NO: 64 - DNA, 27 bp, Mus musculus
aataaggattactatcctatggactac

SEQ ID NO: 65 - protein, 117 aa, Homo sapiens
QVQLVQSGAEVKKPGASVKVSCKASGYTFTKYVIHWVRQAPGQGLEWMGYINPYNDVSKYNEKFRGRVTMTTDTSTSTAYMELRSLRSDDTAVYYCARNKDYYPMDYWGQGTTVTVS

SEQ ID NO: 66 - protein, 5 aa, Mus musculus
KYVIH

SEQ ID NO: 67 - protein, 17 aa, Mus musculus
YINPYNDVSKYNEKFRG

SEQ ID NO: 68 - protein, 9 aa, Mus musculus
NKDYYPMDY

SEQ ID NO: 69 - protein, 11 aa, Mus musculus
SASSSVRFIHW

SEQ ID NO: 70 - protein, 7 aa, Mus musculus
DTSKLAS

SEQ ID NO: 71 - protein, 9 aa, Mus musculus
QQWSSSPFT

SEQ ID NO: 72 - protein, 6 aa, Mus musculus
DYYIHW

SEQ ID NO: 73 - protein, 17 aa, Mus musculus
WIDPENGDTEFVPKFQG

SEQ ID NO: 74 - protein, 4 aa, Mus musculus
TGGF

SEQ ID NO: 75 - protein, 10 aa, Homo sapiens
KPLPEVTDEY

SEQ ID NO: 76 - protein, 18 aa, Homo sapiens
EKEALKKIIEDQQESLNK

SEQ ID NO: 77 - protein, 408 aa, Homo sapiens
MAENGDNEKMAALEAKICHQIEYYFGDFNLPRDKFLKEQIKLDEGWVPLEIMIKFNRLNRLTTDFNVIVEALSKSKAELMEISEDKTKIRRSPSKPLPEVTDEYKNDVKNRSVYIKGFPTDATLDDIKEWLEDKGQVLNIQMRRTLHKAFKGSIFVVFDSIESAKKFVETPGQKYKETDLLILFKDDYFAKKNEERKQNKVEAKLRAKQEQEAKQKLEEDAEMKSLEEKIGCLLKFSGDLDDQTCREDLHILFSNHGEIKWIDFVRGAKEGIILFKEKAKEALGKAKDANNGNLQLRNKEVTWEVLEGEVEKEALKKIIEDQQESLNKWKSKGRRFKGKGKGNKAAQPGSGKGKVQFQGKKTKFASDDEHDEHDENGATGPVKRAREETDKEEPASKQQKTENGAGDQ

SEQ ID NO: 78 - protein, 17 aa, Mus musculus
KSSQSLLNSRTPKNYLA

SEQ ID NO: 79 - protein, 7 aa, Mus musculus
WASTRKS

SEQ ID NO: 80 - protein, 8 aa, Mus musculus
KQSYNLLT

SEQ ID NO: 81 - protein, 5 aa, Mus musculus
HYYIY

SEQ ID NO: 82 - protein, 17 aa, Mus musculus
GVNPSNGGTHFNEKFKS

SEQ ID NO: 83 - protein, 11 aa, Mus musculus
SEYDYGLGFAY

SEQ ID NO: 84 - protein, 17 aa, Mus musculus
RSSQSLLDSRTRKNYLA

SEQ ID NO: 85 - protein, 7 aa, Mus musculus
WASTRES

SEQ ID NO: 86 - protein, 8 aa, Mus musculus
KQSYNLPT

SEQ ID NO: 87 - protein, 5 aa, Mus musculus
DFWMN

SEQ ID NO: 88 - protein, 19 aa, Mus musculus
QIRNKPNNYETYYSDSLKG

SEQ ID NO: 89 - protein, 8 aa, Mus musculus
LGNSWFAY

SEQ ID NO: 90 - DNA, 34 bp, Artificial Sequence
  Primer
  misc_feature (17)..(17): n is a, c, g, or t
tttttggatccsargtnmagctgsagsagtcwgg

SEQ ID NO: 91 - DNA, 30 bp, Artificial Sequence
  Primer
ggaagatctatagacagatgggggtgtcgt

SEQ ID NO: 92 - DNA, 36 bp, Artificial Sequence
  Primer
tttttgaattctgayattgtgmtsacmcarwctmca

SEQ ID NO: 93 - DNA, 32 bp, Artificial Sequence
  Primer
tttttgggcccggatacagttggtgcagcatc

SEQ ID NO: 94 - DNA, 51 bp, Artificial Sequence
  Primer
ggcccagccggccatggcggactacaaagaagtacagctgcaggagtcagg

SEQ ID NO: 95 - DNA, 50 bp, Artificial Sequence
  Primer
ggagccgccgccgccagaaccaccaccacctgaggagacggtgaccgtgg

SEQ ID NO: 96 - DNA, 53 bp, Artificial Sequence
  Primer
ggcggcggcggctccggtggtggtggatccgatattgtgatgacacagtctac

SEQ ID NO: 97 - DNA, 29 bp, Artificial Sequence
  Primer
gcggccgcggatacagttggtgcagcatc

SEQ ID NO: 98 - DNA, 39 bp, Artificial Sequence
  Primer
gggcccgaattcatggcggactacaaagaggtgcagctg

SEQ ID NO: 99 - DNA, 39 bp, Artificial Sequence
  Primer
gggcccaagcttggatacagttggtgcagcatcagcccg

SEQ ID NO: 100 - DNA, 100 bp, Artificial Sequence
  Oligonukleotid
caggttcagctggtgcagtctggagctgaggtgaagaagcctggggcctcagtgaaggtctcctgtaaggcttctggttacacctttaccaaatatgtta

SEQ ID NO: 101 - DNA, 100 bp, Artificial Sequence
  Oligonukleotid
acatcattgtaaggattaatatatcccatccactcaagcccttgtccaggggcctgtcgcacccaatgtataacatatttggtaaaggtgtaaccagaag

SEQ ID NO: 102 - DNA, 100 bp, Artificial Sequence
  Oligonukleotid
gatgggatatattaatccttacaatgatgttagtaagtacaatgagaagttcagaggcagagtcaccatgaccacagacacatccacgagcacagcctac

SEQ ID NO: 103 - DNA, 100 bp, Artificial Sequence
  Oligonukleotid
gatagtaatccttatttctcgcacagtaatacacggccgtgtcgtcagatctcaggctcctcagctccatgtaggctgtgctcgtggatgtgtctgtggt

SEQ ID NO: 104 - DNA, 86 bp, Artificial Sequence
  Oligonukleotid
attactgtgcgagaaataaggattactatcctatggactactggggccaagggaccacggtcaccgtctcgggaggaggaggatcc

SEQ ID NO: 105 - DNA, 37 bp, Artificial Sequence
  Primer
ggcccagccggcccaggttcagctggtgcagtctgga

SEQ ID NO: 106 - DNA, 39 bp, Artificial Sequence
  Primer
ggatcctcctcctcccgagacggtgaccgtggtcccttg

SEQ ID NO: 107 - DNA, 90 bp, Artificial Sequence
  Oligonukleotid
gaaattgtgttgacacagtctccagccaccctgtctttgtctccaggggaaagagccaccctctcctgcagtgccagttcaagtgtaagt

SEQ ID NO: 108 - DNA, 91 bp, Artificial Sequence
  Oligonukleotid
tgtgtcatagatgaggagcctgggagcctggccaggtttctgttggtaccagtgcatgtaacttacacttgaactggcactgcaggagagg

SEQ ID NO: 109 - DNA, 91 bp, Artificial Sequence
  Oligonukleotid
ccaggctcccaggctcctcatctatgacacatccaaactggcttctggcatcccagccaggttcagtggcagtgggtctgggacagacttc

SEQ ID NO: 110 - DNA, 91 bp, Artificial Sequence
  Oligonukleotid
ccactgctgacagtaataaactgcaaaatcttcaggctctaggctgctgatggtgagagtgaagtctgtcccagacccactgccactgaac

SEQ ID NO: 111 - DNA, 79 bp, Artificial Sequence
  Oligonukleotid
agattttgcagtttattactgtcagcagtggagtagtaacccgctcacgttcggcggagggaccaaggtggagatcaaa

SEQ ID NO: 112 - DNA, 27 bp, Artificial Sequence
  Primer
ggatccgaaattgtgttgacacagtct

SEQ ID NO: 113 - DNA, 29 bp, Artificial Sequence
  Primer
gcggccgctttgatctccaccttggtccc

SEQ ID NO: 114 - DNA, 50 bp, Artificial Sequence
  Primer
ggatccgccgccgccagaaccaccaccaccggagcctcctcctcccgaga

SEQ ID NO: 115 - DNA, 100 bp, Artificial Sequence
  Oligonukleotid
gatatccagatgactcaaagtcctagttccctgtctgcatcagtgggagaccgggtgaccattacatgcggtacatcccaagacatcaataattatctca

SEQ ID NO: 116 - DNA, 100 bp, Artificial Sequence
  Oligonukleotid
cggaatgcagcctggatgtgtagtagattaataacttaggaactttgcctggcttctgctgataccagttgagataattattgatgtcttgggatgtacc

SEQ ID NO: 117 - DNA, 100 bp, Artificial Sequence
  Oligonukleotid
aatctactacacatccaggctgcattccggggtgccctcccgcttttcgggctccgggtcgggaaccgactttaccctaaccatatcttccctgcagcct

SEQ ID NO: 118 - DNA, 111 bp, Artificial Sequence
  Oligonukleotid
aagtacagtgagttgcgtcccaccaccaaatgtccatggtaatgtctttgactgctgacaatagtacgttgcaacgtcttcaggctgcagggaagatatggttagggtaaa

SEQ ID NO: 119 - DNA, 29 bp, Artificial Sequence
  Primer
ctcgaggagatatccagatgactcaaagt

SEQ ID NO: 120 - DNA, 57 bp, Artificial Sequence
  Primer
agcggcacttgctccgctccctcctccaccactgccacctccaccaagtacagtgag

SEQ ID NO: 121 - DNA, 100 bp, Artificial Sequence
  Oligonukleotid
caggtgcagctagtggagtccggtggcggcctcgttaagccgggcggatcgctgcgcctttcatgtgccgcatcaggattcacattctccagttactcta

SEQ ID NO: 122 - DNA, 100 bp, Artificial Sequence
  Oligonukleotid
cttccacctgaatcattaatgtacgagacccattccaatcccttgccaggtgcctgccgaatccatgacatagagtaactggagaatgtgaatcctgatg

SEQ ID NO: 123 - DNA, 100 bp, Artificial Sequence
  Oligonukleotid
ggtctcgtacattaatgattcaggtggaagtacattctatccggacacggttaaaggtagatttaccatcagccgtgataacgcgaagaatagcttgtac

SEQ ID NO: 124 - DNA, 100 bp, Artificial Sequence
  Oligonukleotid
tgccataatacatacgtcgagcgcaataatatacagcagtatcctctgcacgcaggctattcatctgtaagtacaagctattcttcgcgttatcacggct

SEQ ID NO: 125 - DNA, 86 bp, Artificial Sequence
  Oligonukleotid
attattgcgctcgacgtatgtattatggcaatagtcactggcactttgacgtctggggccagggcacgacagttactgtctcttcg

SEQ ID NO: 126 - DNA, 58 bp, Artificial Sequence
  Primer
ggagcaagtgccgctggaggcggaggttcaggcggtggtggaagccaggtgcagctag

SEQ ID NO: 127 - DNA, 27 bp, Artificial Sequence
  Primer
gggccccgaagagacagtaactgtcgt

SEQ ID NO: 128 - DNA, 29 bp, Artificial Sequence
  Primer
ctcgaggagatatccagatgactcaaagt

SEQ ID NO: 129 - DNA, 27 bp, Artificial Sequence
  Primer
gggccccgaagagacagtaactgtcgt

SEQ ID NO: 130 - protein, 25 aa, Artificial Sequence
  Peptid
GGGGSGGGGSGASAAGGGGSGGGGS

SEQ ID NO: 131 - protein, 15 aa, Artificial Sequence
  Peptid
GGGGSGGGGSGGGGS

SEQ ID NO: 132 - protein, 5 aa, Artificial Sequence
  Peptid
GGGGS

SEQ ID NO: 133 - protein, 5 aa, Artificial Sequence
  Peptid
AAARG

SEQ ID NO: 134 - DNA, 40 bp, Artificial Sequence
  Primer
ggcccagccggccggatccgatatccagatgactcaaagt

SEQ ID NO: 135 - DNA, 41 bp, Artificial Sequence
  Primer
gcggccgcggatcctcctcctcccgaagagacagtaactgt

SEQ ID NO: 136 - DNA, 39 bp, Artificial Sequence
  Oligonukleotid
ggccgctaaacccctacctgaagtgactgatgagtatgc

SEQ ID NO: 137 - DNA, 39 bp, Artificial Sequence
  Oligonukleotid
tcgagcatactcatcagtcacttcaggtaggggtttagc

SEQ ID NO: 138 - DNA, 100 bp, Artificial Sequence
  Oligonukleotid
caagtgcaactggtccagtcaggtgctgaggtgaaaaaacccggagccagtgtcaaagtaagctgcaaggcctctgggtatactttcacccattactata

SEQ ID NO: 139 - DNA, 100 bp, Artificial Sequence
  Oligonukleotid
ccaccgttcgaagggttgactccacccatccactcaagcccctgacctggagcttgacgaacccagtatatatagtaatgggtgaaagtatacccagagg

SEQ ID NO: 140 - DNA, 100 bp, Artificial Sequence
  Oligonukleotid
gatgggtggagtcaacccttcgaacggtggcactcacttcaatgaaaagtttaaaagccgcgtaaccatgacgcgagatacttccatttccacagcttat

SEQ ID NO: 141 - DNA, 100 bp, Artificial Sequence
  Oligonukleotid
cataatcatattcacttctagcacagtaataaacggccgtgtcatcactgcgtaacctactaagttccatataagctgtggaaatggaagtatctcgcgt

SEQ ID NO: 142 - DNA, 80 bp, Artificial Sequence
  Oligonukleotid
attactgtgctagaagtgaatatgattatgggttgggtttcgcttactggggccagggaaccctcgtcaccgtgtccagt

SEQ ID NO: 143 - DNA, 33 bp, Artificial Sequence
  Primer
ctcgaggacaagtgcaactggtccagtcaggtg

SEQ ID NO: 144 - DNA, 55 bp, Artificial Sequence
  Primer
agaaccgccaccaccggatcctccaccaccactggacacggtgacgagggttccc

SEQ ID NO: 145 - DNA, 100 bp, Artificial Sequence
  Oligonukleotid
gacattgttatgacgcagagccctgattcactcgcagtgtccctaggagagcgggccaccatcaactgtaaaagttctcagtccctgctgaacagcagga

SEQ ID NO: 146 - DNA, 100 bp, Artificial Sequence
  Oligonukleotid
gcccagtaaatgagcagcttaggcggctgtccaggtttctgttggtaccatgccaggtaattcttaggcgtcctgctgttcagcagggactgagaacttt

SEQ ID NO: 147 - DNA, 100 bp, Artificial Sequence
  Oligonukleotid
acagccgcctaagctgctcatttactgggcctccacacggaagagcggcgtgcccgaccggttttccgggagcggctccggcaccgactttaccttgacc

SEQ ID NO: 148 - DNA, 100 bp, Artificial Sequence
  Oligonukleotid
caaatgtcaggagattgtaagattgcttgcaatagtatacggccacgtcttctgcctgcagggaactgatggtcaaggtaaagtcggtgccggagccgct

SEQ ID NO: 149 - DNA, 56 bp, Artificial Sequence
  Oligonukleotid
gcaagcaatcttacaatctcctgacatttggcggcggcacaaaagtggagatcaaa

SEQ ID NO: 150 - DNA, 55 bp, Artificial Sequence
  Primer
ggtggtggcggttctggcggaggcggatccgacattgttatgacgcagagccctg

SEQ ID NO: 151 - DNA, 31 bp, Artificial Sequence
  Primer
gggccctttgatctccacttttgtgccgccg

SEQ ID NO: 152 - DNA, 33 bp, Artificial Sequence; identical to SEQ ID NO: 143
  Primer

SEQ ID NO: 153 - DNA, 31 bp, Artificial Sequence; identical to SEQ ID NO: 151
  Primer

SEQ ID NO: 154 - DNA, 72 bp, Artificial Sequence
  Oligonukleotid
ggccgctctggagaaagaagcactgaagaaaataatagaagaccaacaagaatccctaaacaaagcagctgc

SEQ ID NO: 155 - DNA, 72 bp, Artificial Sequence
  Oligonukleotid
tcgagcagctgctttgtttagggattcttgttggtcttctattattttcttcagtgcttctttctccagagc

SEQ ID NO: 156 - DNA, 100 bp, Artificial Sequence
  Oligonukleotid
gaggtgcaactggtcgaaagtggcggtggtttagttcagcctggtggaagtctacggcttagctgcgcagcatccggtttcacctttagcgacttttgga

SEQ ID NO: 157 - DNA, 100 bp, Artificial Sequence
  Oligonukleotid
ttattcggtttgttgcggatttgcccaacccactccagtcctttgcccggagcctgccgaacccagttcatccaaaagtcgctaaaggtgaaaccggatg

SEQ ID NO: 158 - DNA, 100 bp, Artificial Sequence
  Oligonukleotid
ggttgggcaaatccgcaacaaaccgaataactacgaaacttattactcagatagcctgaagggtcgattcaccatcagcagggatgattcaaagtcaatc

SEQ ID NO: 159 - DNA, 100 bp, Artificial Sequence
  Oligonukleotid
aggagttacctagtgtacagtaatacaccgcagtatcctccgctcttaatgagttcatctgtaggtaagtgattgactttgaatcatccctgctgatggt

SEQ ID NO: 160 - DNA, 74 bp, Artificial Sequence
  Oligonukleotid
cggtgtattactgtacactaggtaactcctggttcgcgtattggggacagggcacccttgtaaccgtctccagc

SEQ ID NO: 161 - DNA, 65 bp, Artificial Sequence
  Primer
ggtggcggcggctccggaggtggtggttccggcggtggcggatcggaggtgcaactggtcgaaag

SEQ ID NO: 162 - DNA, 27 bp, Artificial Sequence
  Primer
gggcccgctggagacggttacaagggt

SEQ ID NO: 163 - DNA, 100 bp, Artificial Sequence
  Oligonukleotid
gacattgttatgacccagagcccggactctctcgctgttagtcttggtgagcgagcgactattaactgccggagcagtcagagtttgttggactcacgga

SEQ ID NO: 164 - DNA, 100 bp, Artificial Sequence
  Oligonukleotid
gcccaatatatcagtaatttaggtggttggcccggcttctgctggtaccatgccaggtagttctttctcgtccgtgagtccaacaaactctgactgctcc

SEQ ID NO: 165 - DNA, 100 bp, Artificial Sequence
  Oligonukleotid
ccaaccacctaaattactgatatattgggcgtcgactcgtgagtcaggggtaccggacaggttttctggaagcggatcaggaacagacttcactttgacg

SEQ ID NO: 166 - DNA, 100 bp, Artificial Sequence
  Oligonukleotid
caaatgtcggcagattatagctttgcttacaataataaaccgcaacgtcctcggcttgaagcgaagagatcgtcaaagtgaagtctgttcctgatccgct

SEQ ID NO: 167 - DNA, 56 bp, Artificial Sequence
  Oligonukleotid
gtaagcaaagctataatctgccgacatttggtggcggcaccaaggttgaaattaag

SEQ ID NO: 168 - DNA, 29 bp, Artificial Sequence
  Primer
ctcgaggagacattgttatgacccagagc

SEQ ID NO: 169 - DNA, 65 bp, Artificial Sequence
  Primer
ggagccgccgccaccggaaccgccgccgccagatcctccgccgcccttaatttcaaccttggtgc

SEQ ID NO: 170 - DNA, 29 bp, Artificial Sequence
  Primer
ctcgaggagacattgttatgacccagagc

SEQ ID NO: 171 - DNA, 27 bp, Artificial Sequence
  Primer
gggcccgctggagacggttacaagggt

SEQ ID NO: 172 - protein, 5 aa, Artificial Sequence
  Peptid
MADYK